European Patent Application EP 4 379 057 A1, published June 5, 2024. Title: Vector system for transformation of Chlorella vulgaris. Applicant: Green Mineral Inc. The sequence listing filed with the application follows.

SEQUENCE LISTING (7 sequences)

SEQ ID NO: 1 - DNA, 4686 bp, Artificial Sequence
  Pka650
agctgataccgctcgccgcagccgaacgaccgagcgcagcgagtcagtgagcgaggaagcggaagagcgcccaatacgcaaaccgcctctccccgcgcgttggccgattcattaatgcagctggcacgacaggtttcccgactggaaagcgggcagtgagcgcaacgcaattaatgtgagttagctcactcattaggcaccccaggctttacactttatgcttccggctcgtatgttgtgtggaattgtgagcggataacaatttcacacaggaaacagctatgaccatgattacgccaagctcgaaattaaccctcactaaagggaacaaaagctggagctccaccgcggtggcggccgctctagaactagtggatcccccgggctgcaggaattcgatatcaagcttatcgataccgtcgacctcgagatttaaatcatgcagtacttgattctatgcatttagagcatgcagattataaacacactgctcttctcagggcgcacccatgatggtgttatattgcgatgtaatagaagtaagcacgatgactggtcatgtacctcaggtaaaggctatttactgggcatatgagcctgagcatatacaaatttaagttcaatatccaagtttacccggtccagcacaagctaacgtatgctgccgcatagcgcctgtgccatcatgatggtcataccccgtgtcggcgcgttttattgcgtaatgcatgatgtaccgcccctgccaggcagtgccagcgctgggttcttatatatcttgtaaacctacacggcaattcaatgaagttcagacgtgatgctcattaattataatggcagtgtccacactgtggactccacagtgtggagtcaactccacaccggtgctaggtatgcaaggatttagtgggcaaaagcttgctgcaaaattaagggcaaaagaattagacaggcagctgtcagcctcagacctgagatctgtatgcaaatattgaagacttcagttgtgcttaccgtggcacacagtgcacagactgtgcgtggcttaaatgcatgcatgcaaaagtaatattgatatcattgatattcttacacgtgcacgctaatcctgtcaggtggcaagatgcgtctgcagactatcatggcattcatatgactgtagaagctcggagcttctgcagtcccaggcaagtcttactcgagtcaatgagagtcggagtcaagtgagaggcaagcttgcaatctgtacccgctggtgcaagactataccccaattttgctcagttgacctgatatctagcggacatgcaccccacccatccatgcataagcgcttcacgtgcatttcacagtgcaaaatggggaaccttctggagcacgggtagcgctgtttgatgcaacgctgccacgactgtccatcactcgtttcagggagggttccttcccttgaccagggggtcgatacgtctctaattctggtggtgcttatccactgtcgagagggataagttccagcgccgctcagagttccatccctcatttccagcgcaagaacagccttagcaactttcgatccctacaacttcagtgcaatggccaagttgaccagtgccgttccggtgctcaccgcgcgcgacgtcgccggagcggtcgagttctggaccgaccggctcgggttctcccgggacttcgtggaggacgacttcgccggtgtggtccgggacgacgtgaccctgttcatcagcgcggtccaggaccaggtggtgccggacaacaccctggcctgggtgtgggtgcgcggcctggacgagctgtacgccgagtggtcggaggtcgtgtccacgaacttccgggacgcctccgggccggccatgaccgagatcggcgagcagccgtgggggcgggagttcgccctgcgcgacccggccggcaactgcgtgcacttcgtggccgaggagcaggactgatcggctgcacaacgcaattagaaagacctcagtactgtaaatcattagcgaacctttaaacctgcagattccctgtggcttagctgctccaaggaatagtactttcaagactgggggtgcctgcttgtgattgctgaactgttggtccatggattgtcccattgtctgtgagcacatgctccacttccacctgtattggcggtacccaattcgccctatagtgagtcgtattacaattcactggccgtcgttttacaacgtcgtgactgggaaaaccctggcgttacccaacttaatcgccttgcagcacatccccctttcgccagctggcgtaatagcgaagaggcccgcaccgatcgcccttcccaacagttgcgcagcctgaatggcgaatggaaattgtaagcgttaatattttgttaaaattcgcgttaaatttttgttaaatcagctcattttttaaccaataggccgaaatcggcaaaatcccttataaatcaaaagaatagaccgagatagggttgagtgttgttccagtttggaacaagagtccactattaaagaacgtggactccaacgtcaaagggcgaaaaaccgtctatcagggcgatggcccactacgtgaaccatcaccctaatcaagttttttggggtcgaggtgccgtaaagcactaaatcggaaccctaaagggagcccccgatttagagcttgacggggaaagccggcgaacgtggcgagaaaggaagggaagaaagcgaaaggagcgggcgctagggcgctggcaagtgtagcggtcacgctgcgcgtaaccaccacacccgccgcgcttaatgcgccgctacagggcgcgtcaggtggcacttttcggggaaatgtgcgcggaacccctatttgtttatttttctaaatacattcaaatatgtatccgctcatgagacaataaccctgataaatgcttcaataatattgaaaaaggaagagtatgagtattcaacatttccgtgtcgcccttattcccttttttgcggcattttgccttcctgtttttgctcacccagaaacgctggtgaaagtaaaagatgctgaagatcagttgggtgcacgagtgggttacatcgaactggatctcaacagcggtaagatccttgagagttttcgccccgaagaacgttttccaatgatgagcacttttaaagttctgctatgtggcgcggtattatcccgtattgacgccgggcaagagcaactcggtcgccgcatacactattctcagaatgacttggttgagtactcaccagtcacagaaaagcatcttacggatggcatgacagtaagagaattatgcagtgctgccataaccatgagtgataacactgcggccaacttacttctgacaacgatcggaggaccgaaggagctaaccgcttttttgcacaacatgggggatcatgtaactcgccttgatcgttgggaaccggagctgaatgaagccataccaaacgacgagcgtgacaccacgatgcctgtagcaatggcaacaacgttgcgcaaactattaactggcgaactacttactctagcttcccggcaacaattaatagactggatggaggcggataaagttgcaggaccacttctgcgctcggcccttccggctggctggtttattgctgataaatctggagccggtgagcgtgggtctcgcggtatcattgcagcactggggccagatggtaagccctcccgtatcgtagttatctacacgacggggagtcaggcaactatggatgaacgaaatagacagatcgctgagataggtgcctcactgattaagcattggtaactgtcagaccaagtttactcatatatactttagattgatttaaaacttcatttttaatttaaaaggatctaggtgaagatcctttttgataatctcatgaccaaaatcccttaacgtgagttttcgttccactgagcgtcagaccccgtagaaaagatcaaaggatcttcttgagatcctttttttctgcgcgtaatctgctgcttgcaaacaaaaaaaccaccgctaccagcggtggtttgtttgccggatcaagagctaccaactctttttccgaaggtaactggcttcagcagagcgcagataccaaatactgtccttctagtgtagccgtagttaggccaccacttcaagaactctgtagcaccgcctacatacctcgctctgctaatcctgttaccagtggctgctgccagtggcgataagtcgtgtcttaccgggttggactcaagacgatagttaccggataaggcgcagcggtcgggctgaacggggggttcgtgcacacagcccagcttggagcgaacgacctacaccgaactgagatacctacagcgtgagctatgagaaagcgccacgcttcccgaagggagaaaggcggacaggtatccggtaagcggcagggtcggaacaggagagcgcacgagggagcttccagggggaaacgcctggtatctttatagtcctgtcgggtttcgccacctctgacttgagcgtcgatttttgtgatgctcgtcaggggggcggagcctatggaaaaacgccagcaacgcggcctttttacggttcctggccttttgctggccttttgctcacatgttctttcctgcgttatcccctgattctgtggataaccgtattaccgcctttgagtg

SEQ ID NO: 2 - DNA, 50 bp, Artificial Sequence
  Promoter
atgcagattataaacacactgctcttctcagggcgcacccatgatggtgt

SEQ ID NO: 3 - DNA, 198 bp, Artificial Sequence
  Terminator
cacaacgcaattagaaagacctcagtactgtaaatcattagcgaacctttaaacctgcagattccctgtggcttagctgctccaaggaatagtactttcaagactgggggtgcctgcttgtgattgctgaactgttggtccatggattgtcccattgtctgtgagcacatgctccacttccacctgtattggcggtac

SEQ ID NO: 4 - DNA, 375 bp, Artificial Sequence
  selectable marker
atggccaagttgaccagtgccgttccggtgctcaccgcgcgcgacgtcgccggagcggtcgagttctggaccgaccggctcgggttctcccgggacttcgtggaggacgacttcgccggtgtggtccgggacgacgtgaccctgttcatcagcgcggtccaggaccaggtggtgccggacaacaccctggcctgggtgtgggtgcgcggcctggacgagctgtacgccgagtggtcggaggtcgtgtccacgaacttccgggacgcctccgggccggccatgaccgagatcggcgagcagccgtgggggcgggagttcgccctgcgcgacccggccggcaactgcgtgcacttcgtggccgaggagcaggactga

SEQ ID NO: 5 - DNA, 18 bp, Artificial Sequence
  Forward primer
atggccaagttgaccagt

SEQ ID NO: 6 - DNA, 20 bp, Artificial Sequence
  Reverse primer
tcagtcctgctcctcggcca

SEQ ID NO: 7 - DNA, 6742 bp, Artificial Sequence
  pJG002
agctgataccgctcgccgcagccgaacgaccgagcgcagcgagtcagtgagcgaggaagcggaagagcgcccaatacgcaaaccgcctctccccgcgcgttggccgattcattaatgcagctggcacgacaggtttcccgactggaaagcgggcagtgagcgcaacgcaattaatgtgagttagctcactcattaggcaccccaggctttacactttatgcttccggctcgtatgttgtgtggaattgtgagcggataacaatttcacacaggaaacagctatgaccatgattacgccaagctcgaaattaaccctcactaaagggaacaaaagctggagctccaccgcggtggcggccgctctagaactagtggatcccccgggctgcaggaattcgatatcaagcttatcgataccgtcgacctcgagatttaaatcatgcagtacttgattctatgcatttagagcatgcagattataaacacactgctcttctcagggcgcacccatgatggtgttatattgcgatgtaatagaagtaagcacgatgactggtcatgtacctcaggtaaaggctatttactgggcatatgagcctgagcatatacaaatttaagttcaatatccaagtttacccggtccagcacaagctaacgtatgctgccgcatagcgcctgtgccatcatgatggtcataccccgtgtcggcgcgttttattgcgtaatgcatgatgtaccgcccctgccaggcagtgccagcgctgggttcttatatatcttgtaaacctacacggcaattcaatgaagttcagacgtgatgctcattaattataatggcagtgtccacactgtggactccacagtgtggagtcaactccacaccggtgctaggtatgcaaggatttagtgggcaaaagcttgctgcaaaattaagggcaaaagaattagacaggcagctgtcagcctcagacctgagatctgtatgcaaatattgaagacttcagttgtgcttaccgtggcacacagtgcacagactgtgcgtggcttaaatgcatgcatgcaaaagtaatattgatatcattgatattcttacacgtgcacgctaatcctgtcaggtggcaagatgcgtctgcagactatcatggcattcatatgactgtagaagctcggagcttctgcagtcccaggcaagtcttactcgagtcaatgagagtcggagtcaagtgagaggcaagcttgcaatctgtacccgctggtgcaagactataccccaattttgctcagttgacctgatatctagcggacatgcaccccacccatccatgcataagcgcttcacgtgcatttcacagtgcaaaatggggaaccttctggagcacgggtagcgctgtttgatgcaacgctgccacgactgtccatcactcgtttcagggagggttccttcccttgaccagggggtcgatacgtctctaattctggtggtgcttatccactgtcgagagggataagttccagcgccgctcagagttccatccctcatttccagcgcaagaacagccttagcaactttcgatccctacaacttcagtgcaatggccaagttgaccagtgccgttccggtgctcaccgcgcgcgacgtcgccggagcggtcgagttctggaccgaccggctcgggttctcccgggacttcgtggaggacgacttcgccggtgtggtccgggacgacgtgaccctgttcatcagcgcggtccaggaccaggtggtgccggacaacaccctggcctgggtgtgggtgcgcggcctggacgagctgtacgccgagtggtcggaggtcgtgtccacgaacttccgggacgcctccgggccggccatgaccgagatcggcgagcagccgtgggggcgggagttcgccctgcgcgacccggccggcaactgcgtgcacttcgtggccgaggagcaggactgatcggctgcacaacgcaattagaaagacctcagtactgtaaatcattagcgaacctttaaacctgcagattccctgtggcttagctgctccaaggaatagtactttcaagactgggggtgcctgcttgtgattgctgaactgttggtccatggattgtcccattgtctgtgagcacatgctccacttccacctgtattggcggtaccaaatcatgcagtacttgattctatgcatttagagcatgcagattataaacacactgctcttctcagggcgcacccatgatggtgttatattgcgatgtaatagaagtaagcacgatgactggtcatgtacctcaggtaaaggctatttactgggcatatgagcctgagcatatacaaatttaagttcaatatccaagtttacccggtccagcacaagctaacgtatgctgccgcatagcgcctgtgccatcatgatggtcataccccgtgtcggcgcgttttattgcgtaatgcatgatgtaccgcccctgccaggcagtgccagcgctgggttcttatatatcttgtaaacctacacggcaattcaatgaagttcagacgtgatgctcattaattataatggcagtgtccacactgtggactccacagtgtggagtcaactccacaccggtgctaggtatgcaaggatttagtgggcaaaagcttgctgcaaaattaagggcaaaagaattagacaggcagctgtcagcctcagacctgagatctgtatgcaaatattgaagacttcagttgtgcttaccgtggcacacagtgcacagactgtgcgtggcttaaatgcatgcatgcaaaagtaatattgatatcattgatattcttacacgtgcacgctaatcctgtcaggtggcaagatgcgtctgcagactatcatggcattcatatgactgtagaagctcggagcttctgcagtcccaggcaagtcttactcgagtcaatgagagtcggagtcaagtgagaggcaagcttgcaatctgtacccgctggtgcaagactataccccaattttgctcagttgacctgatatctagcggacatgcaccccacccatccatgcataagcgcttcacgtgcatttcacagtgcaaaatggggaaccttctggagcacgggtagcgctgtttgatgcaacgctgccacgactgtccatcactcgtttcagggagggttccttcccttgaccagggggtcgatacgtctctaattctggtggtgcttatccactgtcgagagggataagttccagcgccgctcagagttccatccctcatttccagcgcaagaacagccttagcaactttcgatccctacaacttcagtgcaatggctattgaaggcactacgtctgacattacccctttgctggaggccaatcggaaatgggcggaggagtgcatcgccaaggaccccacctatttctcgaagattgctggctcacagtctccagaattcctctacattggctgctctgactctcgcgcgcacccggccgcgatgttcagcatggcgcccggggaggtgtttgtgcagcgcaacgtcggcaacctgatcagcgtcaaagacctcaactgcatgagctgcctggagtacacaatcgaccacctcaaggtcaagcacatcctcgtcaccggccactacaactgcggtgcgtgcaaggcgggactcgtgtggcacccgagcacggcgggggtgactaacctgtggatctctgatgtgagggacgtgcgtgacaagaacgctgccgctctggagggcctccccctcgacgaagcctgggacaagctggtggaattgaacgtggaggcgcaggtgttcaacgtggtctcgtcgccggtggtgcaggcggcgtgggcgcgcggccagcagctggtggtgcatggactggtttatacccccggcaccggcagggtcaaggagctgatcaagcccgtcacgggcaatgatgacggcacctacagcctgtctgccaaactgaagaagcactgctccttctctgagtccctcaagtgatcggctgcacaacgcaattagaaagacctcagtactgtaaatcattagcgaacctttaaacctgcagattccctgtggcttagctgctccaaggaatagtactttcaagactgggggtgcctgcttgtgattgctgaactgttggtccatggattgtcccattgtctgtgagcacatgctccacttccacctgtattggcggtacgggccccaattcgccctatagtgagtcgtattacaattcactggccgtcgttttacaacgtcgtgactgggaaaaccctggcgttacccaacttaatcgccttgcagcacatccccctttcgccagctggcgtaatagcgaagaggcccgcaccgatcgcccttcccaacagttgcgcagcctgaatggcgaatggaaattgtaagcgttaatattttgttaaaattcgcgttaaatttttgttaaatcagctcattttttaaccaataggccgaaatcggcaaaatcccttataaatcaaaagaatagaccgagatagggttgagtgttgttccagtttggaacaagagtccactattaaagaacgtggactccaacgtcaaagggcgaaaaaccgtctatcagggcgatggcccactacgtgaaccatcaccctaatcaagttttttggggtcgaggtgccgtaaagcactaaatcggaaccctaaagggagcccccgatttagagcttgacggggaaagccggcgaacgtggcgagaaaggaagggaagaaagcgaaaggagcgggcgctagggcgctggcaagtgtagcggtcacgctgcgcgtaaccaccacacccgccgcgcttaatgcgccgctacagggcgcgtcaggtggcacttttcggggaaatgtgcgcggaacccctatttgtttatttttctaaatacattcaaatatgtatccgctcatgagacaataaccctgataaatgcttcaataatattgaaaaaggaagagtatgagtattcaacatttccgtgtcgcccttattcccttttttgcggcattttgccttcctgtttttgctcacccagaaacgctggtgaaagtaaaagatgctgaagatcagttgggtgcacgagtgggttacatcgaactggatctcaacagcggtaagatccttgagagttttcgccccgaagaacgttttccaatgatgagcacttttaaagttctgctatgtggcgcggtattatcccgtattgacgccgggcaagagcaactcggtcgccgcatacactattctcagaatgacttggttgagtactcaccagtcacagaaaagcatcttacggatggcatgacagtaagagaattatgcagtgctgccataaccatgagtgataacactgcggccaacttacttctgacaacgatcggaggaccgaaggagctaaccgcttttttgcacaacatgggggatcatgtaactcgccttgatcgttgggaaccggagctgaatgaagccataccaaacgacgagcgtgacaccacgatgcctgtagcaatggcaacaacgttgcgcaaactattaactggcgaactacttactctagcttcccggcaacaattaatagactggatggaggcggataaagttgcaggaccacttctgcgctcggcccttccggctggctggtttattgctgataaatctggagccggtgagcgtgggtctcgcggtatcattgcagcactggggccagatggtaagccctcccgtatcgtagttatctacacgacggggagtcaggcaactatggatgaacgaaatagacagatcgctgagataggtgcctcactgattaagcattggtaactgtcagaccaagtttactcatatatactttagattgatttaaaacttcatttttaatttaaaaggatctaggtgaagatcctttttgataatctcatgaccaaaatcccttaacgtgagttttcgttccactgagcgtcagaccccgtagaaaagatcaaaggatcttcttgagatcctttttttctgcgcgtaatctgctgcttgcaaacaaaaaaaccaccgctaccagcggtggtttgtttgccggatcaagagctaccaactctttttccgaaggtaactggcttcagcagagcgcagataccaaatactgtccttctagtgtagccgtagttaggccaccacttcaagaactctgtagcaccgcctacatacctcgctctgctaatcctgttaccagtggctgctgccagtggcgataagtcgtgtcttaccgggttggactcaagacgatagttaccggataaggcgcagcggtcgggctgaacggggggttcgtgcacacagcccagcttggagcgaacgacctacaccgaactgagatacctacagcgtgagctatgagaaagcgccacgcttcccgaagggagaaaggcggacaggtatccggtaagcggcagggtcggaacaggagagcgcacgagggagcttccagggggaaacgcctggtatctttatagtcctgtcgggtttcgccacctctgacttgagcgtcgatttttgtgatgctcgtcaggggggcggagcctatggaaaaacgccagcaacgcggcctttttacggttcctggccttttgctggccttttgctcacatgttctttcctgcgttatcccctgattctgtggataaccgtattaccgcctttgagtg